European Patent Specification EP 3 530 669 B1, published October 15, 2025. Title: NON-HEMOLYTIC LLO FUSION PROTEINS AND USES THEREOF. Applicant: The Trustees of the University of Pennsylvania. The sequence listing filed with the application follows.

SEQUENCE LISTING (63 sequences)

SEQ ID NO: 1 - protein, 180 aa, Homo sapiens
MQAEGRGTGGSTGDADGPGGPGIPDGPGGNAGGPGEAGATGGRGPRGAGAARASGPGGGAPRGPHGGAASGLNGCCRCGARGPESRLLEFYLAMPFATPMEAELARRSLAQDAPPLPVPGVLLKEFTVSGNILTIRLTAADHRQLQLSISSCLQQLSLLMWITQCFLPVFLAQPPSGQRR

SEQ ID NO: 2 - protein, 9 aa, Homo sapiens
SLLMWITQC

SEQ ID NO: 3 - protein, 11 aa, Homo sapiens
SLLMWITQCFL

SEQ ID NO: 4 - protein, 12 aa, Homo sapiens
SLLMWITQCFLP

SEQ ID NO: 5 - protein, 13 aa, Homo sapiens
SLLMWITQCFLPV

SEQ ID NO: 6 - protein, 14 aa, Homo sapiens
SLLMWITQCFLPVF

SEQ ID NO: 7 - protein, 15 aa, Homo sapiens
SLLMWITQCFLPVFL

SEQ ID NO: 8 - protein, 20 aa, Homo sapiens
WITQCFLPVFLAQPPSGQRR

SEQ ID NO: 9 - protein, 20 aa, Homo sapiens
YLAMPFATPMEAELARRSLA

SEQ ID NO: 10 - protein, 10 aa, Homo sapiens
ASGPGGGAPR

SEQ ID NO: 11 - protein, 9 aa, Homo sapiens
MPFATPMEA

SEQ ID NO: 12 - protein, 9 aa, Homo sapiens
LAMPFATPM

SEQ ID NO: 13 - protein, 9 aa, Homo sapiens
ARGPESRLL

SEQ ID NO: 14 - protein, 9 aa, Homo sapiens
LLMWITQCF

SEQ ID NO: 15 - protein, 9 aa, Homo sapiens
SLLMWITQV

SEQ ID NO: 16 - protein, 9 aa, Homo sapiens
SLLMWITQV

SEQ ID NO: 17 - protein, 98 aa, Human papillomavirus
MHGDTPTLHEYMLDLQPETTDLYCYEQLNDSSEEEDEIDGPAGQAEPDRAHYNIVTFCCKCDSTLRLCVQSTHVDIRTLEDLLMGTLGIVCPICSQKP

SEQ ID NO: 18 - protein, 11 aa, Listeria monocytogenes
ECTGLAWEWWR

SEQ ID NO: 19 - protein, 9 aa, Human papillomavirus
RAHYNIVTF

SEQ ID NO: 20 - protein, 105 aa, Human papillomavirus
MHGPKATLQDIVLHLEPQNEIPVDLLCHEQLSDSEEENDEIDGVNHQHLPARRAEPQRHTMLCMCCKCEARIELVVESSADDLRAFQQLFLNTLSFVCPWCASQQ

SEQ ID NO: 21 - protein, 8 aa, Human papillomavirus
TLGIVCPI

SEQ ID NO: 22 - protein, 9 aa, Human papillomavirus
LLMGTLGIV

SEQ ID NO: 23 - protein, 10 aa, Human papillomavirus
YMLDLQPETT

SEQ ID NO: 24 - protein, 158 aa, Human papillomavirus
MHQKRTAMFQDPQERPRKLPQLCTELQTTIHDIILECVYCKQQLLRREVYDFAFRDLCIVYRDGNPYAVCDKCLKFYSKISEYRHYCYSLYGTTLEQQYNKPLCDLLIRCINCQKPLCPEEKQRHLDKKQRFHNIRGRWTGRCMSCCRSSRTRRETQL

SEQ ID NO: 25 - protein, 158 aa, Human papillomavirus
MARFEDPTRRPYKLPDLCTELNTSLQDIEITCVYCKTVLELTEVFEFAFKDLFVVYRDSIPHAACHKCIDFYSRIRELRHYSDSVYGDTLEKLTNTGLYNLLIRCLRCQKPLNPAEKLRHLNEKRRFHNIAGHYRGQCHSCCNRARQERLQRRRETQV

SEQ ID NO: 26 - protein, 145 aa, Mus musculus
MKLWLNWIFLVTLLNGIQCEVKLVESGGGLVQPGGSLSLSCAASGFTFTDYYMSWVRQPPGKALEWLALIRNKANGYTTEYSASVKGRFTISRDNSQSILYLQMNALRAEDSATYYCARDPNYYDGSYEGYFDYWAQGTTLTVSS

SEQ ID NO: 27 - protein, 124 aa, Mus musculus
LLLISVTVIVSNGEIVLTQSPTTMAASPGEKITITCSASSSISSNYLHWYQQKPGFSPKLLIYRTSNLASGVPARFSGSGSGTSYSLTIGTMEAEDVATYYCQQGSSIPRGVTFGSGTKLEIKR

SEQ ID NO: 28 - protein, 132 aa, Mus musculus
GFLLISVTVILTNGEIFLTQSPAIIAASPGEKVTITCSASSSVSYMNWYQQKPGSSPKIWIYGISNLASGVPARFSGSGSGTSFSFTINSMEAEDVATYYCQQRSSYPFTFGSGTKLEIKRADAAPTVSHLP

SEQ ID NO: 29 - protein, 123 aa, Mus musculus
LLLISVTVIVSNGEIVLTQSPTTMAASPGEKITITCSASSSISSNYLHWYQQKPGFSPKLLIYRTSNLASGVPARFSGSGSGTSYSLTIGTMEAEDVATYYCQQGSSIPRTFGSGTKLEIKRA

SEQ ID NO: 30 - protein, 157 aa, Homo sapiens
MEFGLSWVFLVAILKGVQCEMQLVESGGGLVQPGESLKLSCAASGFSFSGSTIHWVRQASGRGLEWVGRSRSKADNFMTSYAPSIKGKFIISRDDSSNMLYLQMNNLKTEDTAVYFCTRNFTSLDSTGNSFGPWGQGTLVTVSSGSASAPTLFPLVS

SEQ ID NO: 31 - protein, 157 aa, Homo sapiens
MEFGLSWVFLVAILKGVQCEMQLVESGGGLVQPGESFKLSCAASGFSFSGSTIHWVRQASGRGLEWVGRSRSKADNFMTSYAPSIKGKFIISRDDSSNMMYLQMNNLKNEDTAVYFCTRNFTSLDSTGNSFGPWGQGTLVTVSSGSASAPTLFPLVS

SEQ ID NO: 32 - protein, 146 aa, Homo sapiens
MEFGLSWVFLVAILKGVQCEVQLVESGGGLVQPGGSLRLSCAASGFTVSSNYMSWVRQAPGKGLEWVSVIYSGGSTYYADSVKGRFTISRDNSKNTLYLQMNSLRAEDTAVYYCARHTVRGGHCAPRHKPSLQERWGNQRQGALRS

SEQ ID NO: 33 - protein, 134 aa, Homo sapiens
MEFGLSWVFLVAILKGVQCEVQLVESGGGLVQPGGSLKLSCAASGFTFSGSAMHWVRQASGKGLEWVGHIRDKANSYATTYAASVKGRFTISRDDSKNTAYLQMNSLKIEDTAVYFCTRNFTSLDSTGNSFGPW

SEQ ID NO: 34 - protein, 108 aa, Homo sapiens
SELTQDPVVSVALGQTVRITCQGDSLRSYYASWYQQKPGQAPVLVIYGKNNRPSGIPDRFSGSSSGNTASLTITGAQAEDEADYYCNSRDSSGNLPLFGGGTKLTVLG

SEQ ID NO: 35 - protein, 114 aa, Homo sapiens
DIQMTQSPDSLTVSLGERATINCKSSQSILYSSNDKNYLAWYQQKAGQPPKLLIYWASTRESGVPDRFSGSGSATDFTLTISSLQAEDVAIYYCQQYYSTPLTFGGGTKVEIKR

SEQ ID NO: 36 - protein, 108 aa, Homo sapiens
DIQMTQSPSTLSASVGDRVTITCRASQSISTWLAWYQQKPGKAPKLLIYEASSLESGVPSRFSGSGSGTEFTLTISSLQPDDFVTYYCQQYNTFSSYTFGQGTKVEIK

SEQ ID NO: 37 - protein, 529 aa, Listeria monocytogenes
MKKIMLVFITLILVSLPIAQQTEAKDASAFNKENSISSMAPPASPPASPKTPIEKKHADEIDKYIQGLDYNKNNVLVYHGDAVTNVPPRKGYKDGNEYIVVEKKKKSINQNNADIQVVNAISSLTYPGALVKANSELVENQPDVLPVKRDSLTLSIDLPGMTNQDNKIVVKNATKSNVNNAVNTLVERWNEKYAQAYPNVSAKIDYDDEMAYSESQLIAKFGTAFKAVNNSLNVNFGAISEGKMQEEVISFKQIYYNVNVNEPTRPSRFFGKAVTKEQLQALGVNAENPPAYISSVAYGRQVYLKLSTNSHSTKVKAAFDAAVSGKSVSGDVELTNIIKNSSFKAVIYGGSAKDEVQIIDGNLGDLRDILKKGATFNRETPGVPIAYTTNFLKDNELAVIKNNSEYIETTSKAYTDGKINIDHSGGYVAQFNISWDEVNYDPEGNEIVQHKNWSENNKSKLAHFTSSIYLPGNARNINVYAKECTGLAWEWWRTVIDDRNLPLVKNRNISIWGTTLYPKYSNKVDNPIE

SEQ ID NO: 38 - DNA, 22 bp, Artificial Sequence
  Primer
ggctcgagcatggagatacacc

SEQ ID NO: 39 - DNA, 28 bp, Artificial Sequence
  Primer
ggggactagtttatggtttctgagaaca

SEQ ID NO: 40 - DNA, 31 bp, Artificial Sequence
  Primer
gggggctagccctcctttgattagtatattc

SEQ ID NO: 41 - DNA, 28 bp, Artificial Sequence
  Primer
ctccctcgagatcataatttacttcatc

SEQ ID NO: 42 - DNA, 55 bp, Artificial Sequence
  Primer
gactacaaggacgatgaccgacaagtgataacccgggatctaaataaatccgttt

SEQ ID NO: 43 - DNA, 27 bp, Artificial Sequence
  Primer
cccgtcgaccagctcttcttggtgaag

SEQ ID NO: 44 - DNA, 25 bp, Artificial Sequence
  Primer
gcggatcccatggagatacacctac

SEQ ID NO: 45 - DNA, 22 bp, Artificial Sequence
  Primer
gctctagattatggtttctgag

SEQ ID NO: 46 - protein, 529 aa, Listeria monocytogenes
MKKIMLVFITLILVSLPIAQQTEAKDASAFNKENSISSVAPPASPPASPKTPIEKKHADEIDKYIQGLDYNKNNVLVYHGDAVTNVPPRKGYKDGNEYIVVEKKKKSINQNNADIQVVNAISSLTYPGALVKANSELVENQPDVLPVKRDSLTLSIDLPGMTNQDNKIVVKNATKSNVNNAVNTLVERWNEKYAQAYSNVSAKIDYDDEMAYSESQLIAKFGTAFKAVNNSLNVNFGAISEGKMQEEVISFKQIYYNVNVNEPTRPSRFFGKAVTKEQLQALGVNAENPPAYISSVAYGRQVYLKLSTNSHSTKVKAAFDAAVSGKSVSGDVELTNIIKNSSFKAVIYGGSAKDEVQIIDGNLGDLRDILKKGATFNRETPGVPIAYTTNFLKDNELAVIKNNSEYIETTSKAYTDGKINIDHSGGYVAQFNISWDEVNYDPEGNEIVQHKNWSENNKSKLAHFTSSIYLPGNARNINVYAKECTGLAWEWWRTVIDDRNLPLVKNRNISIWGTTLYPKYSNKVDNPIE

SEQ ID NO: 47 - protein, 535 aa, Listeria monocytogenes
MKKIMLVFITLILVSLPIAQQTEAKDASAFNKENSISSVAPPASPPASPKTPIEKKHADEIDKYIQGLDYNKNNVLVYHGDAVTNVPPRKGYKDGNEYIVVEKKKKSINQNNADIQVVNAISSLTYPGALVKANSELVENQPDVLPVKRDSLTLSIDLPGMTNQDNKIVVKNATKSNVNNAVNTLVERWNEKYAQAYSNVSAKIDYDDEMAYSESQLIAKFGTAFKAVNNSLNVNFGAISEGKMQEEVISFKQIYYNVNVNEPTRPSRFFGKAVTKEQLQALGVNAENPPAYISSVAYGRQVYLKLSTNSHSTKVKAAFDAAVSGKSVSGDVELTNIIKNSSFKAVIYGGSAKDEVQIIDGNLGDLRDILKKGATFNRETPGVPIAYTTNFLKDNELAVIKNNSEYIETTSKAYTDGKINIDHSGGYVAQFNISWDEVNYDPEGNEIVQHKNWSENNKSKLAHFTSSIYLPGNARNINVYAKECTGLAWEWWRTVIDDRNLPLVKNRNISIWGTTLYPKYSNKVDNPIEHHHHHH

SEQ ID NO: 48 - DNA, 1551 bp, Listeria monocytogenes
catatgaaggatgcatctgcattcaataaagaaaattcaatttcatccgtggcaccaccagcatctccgcctgcaagtcctaagacgccaatcgaaaagaaacacgcggatgaaatcgataagtatatacaaggattggattacaataaaaacaatgtattagtataccacggagatgcagtgacaaatgtgccgccaagaaaaggttacaaagatggaaatgaatatattgttgtggagaaaaagaagaaatccatcaatcaaaataatgcagacattcaagttgtgaatgcaatttcgagcctaacctatccaggtgctctcgtaaaagcgaattcggaattagtagaaaatcaaccagatgttctccctgtaaaacgtgattcattaacactcagcattgatttgccaggtatgactaatcaagacaataaaatagttgtaaaaaatgccactaaatcaaacgttaacaacgcagtaaatacattagtggaaagatggaatgaaaaatatgctcaagcttattcaaatgtaagtgcaaaaattgattatgatgacgaaatggcttacagtgaatcacaattaattgcgaaatttggtacagcatttaaagctgtaaataatagcttgaatgtaaacttcggcgcaatcagtgaagggaaaatgcaagaagaagtcattagttttaaacaaatttactataacgtgaatgttaatgaacctacaagaccttccagatttttcggcaaagctgttactaaagagcagttgcaagcgcttggagtgaatgcagaaaatcctcctgcatatatctcaagtgtggcgtatggccgtcaagtttatttgaaattatcaactaattcccatagtactaaagtaaaagctgcttttgatgctgccgtaagcggaaaatctgtctcaggtgatgtagaactaacaaatatcatcaaaaattcttccttcaaagccgtaatttacggaggttccgcaaaagatgaagttcaaatcatcgacggcaacctcggagacttacgcgatattttgaaaaaaggcgctacttttaatcgagaaacaccaggagttcccattgcttatacaacaaacttcctaaaagacaatgaattagctgttattaaaaacaactcagaatatattgaaacaacttcaaaagcttatacagatggaaaaattaacatcgatcactctggaggatacgttgctcaattcaacatttcttgggatgaagtaaattatgatcctgaaggtaacgaaattgttcaacataaaaactggagcgaaaacaataaaagcaagctagctcatttcacatcgtccatctatttgcctggtaacgcgagaaatattaatgtttacgctaaagaatgcactggtttagcttgggaatggtggagaacggtaattgatgaccggaacttaccacttgtgaaaaatagaaatatctccatctggggcaccacgctttatccgaaatatagtaataaagtagataatccaatcgaacaccaccaccaccaccactaataaggatcc

SEQ ID NO: 49 - DNA, 20 bp, Artificial
  Primer
gctagctcatttcacatcgt

SEQ ID NO: 50 - DNA, 54 bp, Artificial
  Primer
tcttgcagcttcccaagctaaaccagtcgcttctttagcgtaaacattaatatt

SEQ ID NO: 51 - DNA, 54 bp, Artificial
  Primer
gaagcgactggtttagcttgggaagctgcaagaacggtaattgatgaccggaac

SEQ ID NO: 52 - DNA, 39 bp, Artificial
  Primer
ggatccttattagtggtggtggtggtggtgttcgattgg

SEQ ID NO: 53 - protein, 11 aa, Listeria monocytogenes
EATGLAWEAAR

SEQ ID NO: 54 - protein, 238 aa, Listeria monocytogenes
GCTAGCTCATTTCACATCGTCCATCTATTTGCCTGGTAACGCGAGAAATATTAATGTTTACGCTAAAGAAGCGACTGGTTTAGCTTGGGAAGCTGCAAGAACGGTAATTGATGACCGGAACTTACCACTTGTGAAAAATAGAAATATCTCCATCTGGGGCACCACGCTTTATCCGAAATATAGTAATAAAGTAGATAATCCAATCGAACACCACCACCACCACCACTAATAAGGATCC

SEQ ID NO: 55 - protein, 11 aa, Listeria monocytogenes
ESLLMWITQCR

SEQ ID NO: 56 - protein, 20 aa, Artificial
  Primer
GCTAGCTCATTTCACATCGT

SEQ ID NO: 57 - protein, 54 aa, Artificial
  Primer
TCTGCACTGGGTGATCCACATCAGCAGGCTTTCTTTAGCGTAAACATTAATATT

SEQ ID NO: 58 - protein, 54 aa, Artificial
  Primer
GAAAGCCTGCTGATGTGGATCACCCAGTGCAGAACGGTAATTGATGACCGGAAC

SEQ ID NO: 59 - protein, 39 aa, Artificial
  Primer
GGATCCTTATTAGTGGTGGTGGTGGTGGTGTTCGATTGG

SEQ ID NO: 60 - protein, 238 aa, Listeria monocytogenes
GCTAGCTCATTTCACATCGTCCATCTATTTGCCTGGTAACGCGAGAAATATTAATGTTTACGCTAAAGAAAGCCTGCTGATGTGGATCACCCAGTGCAGAACGGTAATTGATGACCGGAACTTACCACTTGTGAAAAATAGAAATATCTCCATCTGGGGCACCACGCTTTATCCGAAATATAGTAATAAAGTAGATAATCCAATCGAACACCACCACCACCACCACTAATAAGGATCC

SEQ ID NO: 61 - protein, 810 aa, Homo sapiens
GCCCAGCCGCCATGCCAGGTGAAGCTGCAGGAGTCAGGAGGAGGCTTGGTCCAGCCTGGGGGTTCTCTGAGTCTCTCCTGTGCAGCTTCTGGATTCACCTTCACTGATTACTACATGAGCTGGGTCCGCCAGCCTCCAGGGAAGGCACTTGAGTGGTTGGCTTTGATTAGAAACAAAGCTAATGGTTACACAGAGTACAGTGCATCTGTGAAGGGTCGGTTCACCATCTCCAGAGATAATTCCCAAAGCATCCTCTATCTTCAAATGAATGCCCTGAGAGCTGAGGACAGTGCCACTTATTACTGTGCAAGAGATCCCAATTACTACGATGGTAGCTACGAAGGGTACTTTGACTACTGGGGCCAAGGGACCACGGTCACCGTCTCCTCAGGCGGAGGCGGTTCAGGCGGAGGTGGCTCTGGCGGTGGCGGATCGGACATTGAGCTCACCCAGTCTCCATCCTCACTGTCTGCATCTCTGGGAGGCAAAGTCACCATCACTTGCAAGGCAAGCCAAGACATTAACAAGTATATAGCTTGGTACCAACACAAGCCTGGAAAAGGTCCTAGGCTGCTCATACATTACACATCTACATTACAGCCAGGCATCCCATCAAGGTTCAGTGGAAGTGGGTCTGGGAGAGATTATTCCTTCAGCATCAGCAACCTGGAGCCTGAAGATATTGCAACTTATTATTGTCTACAGTATGATAATCTGTACACGTTCGGCTCGGGGACCAAGCTGGAAATAAAACGGGCGGCCGCAGAACAAAAACTCATCTCAGAAGAGGATCTGAATTAATAAGAATTC

SEQ ID NO: 62 - protein, 285 aa, Homo sapiens
MKYLLPTAAAGLLLLAAQPAQPPCQVKLQESGGGLVQPGGSLSLSCAASGFTFTDYYMSWVRQPPGKALEWLALIRNKANGYTEYSASVKGRFTISRDNSQSILYLQMNALRAEDSATYYCARDPNYYDGSYEGYFDYWGQGTTVTVSSGGGGSGGGGSGGGGSDIELTQSPSSLSASLGGKVTITCKASQDINKYIAWYQHKPGKGPRLLIHYTSTLQPGIPSRFSGSGSGRDYSFSISNLEPEDIATYYCLQYDNLYTFGSGTKLEIKRAAAEQKLISEEDLN

SEQ ID NO: 63 - protein, 32 aa, Listeria monocytogenes
KENSISSMAPPASPPASPKTPIEKKHADEIDK